European Patent Specification EP 3 845 667 B1, published January 14, 2026. Title: METHOD OF AMPLIFYING AND DETERMINING TARGET NUCLEOTIDE SEQUENCE. Applicant: Industrial Technology Research Institute. The sequence listing filed with the application follows.

SEQUENCE LISTING (14 sequences)

SEQ ID NO: 1 - DNA, 12 bp, Artificial Sequence
  Synthetic
gagctcgaattc

SEQ ID NO: 2 - DNA, 12 bp, Artificial Sequence
  Synthetic
ggatcctctaga

SEQ ID NO: 3 - DNA, 100 bp, Artificial Sequence
  Synthetic
aaggtactcgtgctgtatctacaactgagggagctgggtgctgacaccccaaaaggccgcacttttccccttaagagagtaaacttgtttcgaaggcaga

SEQ ID NO: 4 - DNA, 186 bp, Artificial Sequence
  Synthetic
agatgagaaagaaagagtaggcacagagctcgaattcaaggtactcgtgctgtatctacaactgagggagctgggtgctgacaccccaaaaggccgcacttttccccttaagagagtaaacttgtttcgaaggcagaggatcctctagagtctctcgcgcccccttgcctcatctctagaggatcc

SEQ ID NO: 5 - DNA, 137 bp, Artificial Sequence
  Synthetic
tctgccttcgaaacaagtttactctcttaaggggaaaagtgcggccttttggggtgtcagcacccagctccctcagttgtagatacagcacgagtaccttgaattcgagctcttccaaaattggccaaaggctatag

SEQ ID NO: 6 - DNA, 25 bp, Artificial Sequence
  Synthetic
atgagaaagaaagagtaggcacaga

SEQ ID NO: 7 - DNA, 25 bp, Artificial Sequence
  Synthetic
tatagcctttggccaattttggaag

SEQ ID NO: 8 - DNA, 323 bp, Artificial Sequence
  Synthetic
agatgagaaagaaagagtaggcacagagctcgaattcaaggtactcgtgctgtatctacaactgagggagctgggtgctgacaccccaaaaggccgcacttttccccttaagagagtaaacttgtttcgaaggcagaggatcctctagagtctctcgcgcccccttgcctcatctctagaggatcctctgccttcgaaacaagtttactctcttaaggggaaaagtgcggccttttggggtgtcagcacccagctccctcagttgtagatacagcacgagtaccttgaattcgagctcttccaaaattggccaaaggctatag

SEQ ID NO: 9 - DNA, 323 bp, Artificial Sequence
  Synthetic
agatgagaaagaaagagtaggcacagagtttgaatttaaggtattcgtgttgtatttataattgagggagttgggtgttgatattttaaaaggtcgtatttttttttttaagagagtaaatttgtttcgaaggtagaggattttttagagttttttgtgtttttttgttttatttttagaggattttttgtttttgaaataagtttatttttttaaggggaaaagtgtggttttttggggtgttagtatttagtttttttagttgtagatatagtatgagtattttgaatttgagttcttccaaaattggccaaaggctatag

SEQ ID NO: 10 - DNA, 296 bp, Artificial Sequence
  Synthetic
tttttagaaaggaagagtaggccccgagtttgaatttaaggtattcgtgttgtatttataattgagggagttgggtgttgatattttaaaaggtcgtatttttttttttaagagagtaaatttgtttcgaaggtagaggattttttagagttttttgtgtttttttgttttatttttagaggattttttgtttttgaaataagtttatttttttaaggggaaaagtgtggttttttggggtgttagtatttagtttttttagttgtagatatagtatgagtatttgaatttgctgt

SEQ ID NO: 11 - DNA, 323 bp, Artificial Sequence
  Synthetic
ctatagcctttggccaattttggaagagctcgaattcaaggtactcgtgctgtatctacaactgagggagctgggtgctgacaccccaaaaggccgcacttttccccttaagagagtaaacttgtttcgaaggcagaggatcctctagagatgaggcaagggggcgcgagagactctagaggatcctctgccttcgaaacaagtttactctcttaaggggaaaagtgcggccttttggggtgtcagcacccagctccctcagttgtagatacagcacgagtaccttgaattcgagctctgtgcctactctttctttctcatct

SEQ ID NO: 12 - DNA, 323 bp, Artificial Sequence
  Synthetic
ctatagcctttggccaattttggaagaactcaaattcaaaatactcatactatatctacaactaaaaaaactaaatactaacaccccaaaaaaccacacttttccccttaaaaaaataaacttatttcaaaaacaaaaaatcctctaaaaataaaacaaaaaaacacaaaaaactctaaaaaatcctctaccttcgaaacaaatttactctcttaaaaaaaaaaatacgaccttttaaaatatcaacacccaactccctcaattataaatacaacacgaataccttaaattcaaactctgtgcctactctttctttctcatct

SEQ ID NO: 13 - DNA, 299 bp, Artificial Sequence
  Synthetic
gagggcttgatttaggtattcgtgttgtatttataattgagggagttgggtgttgatattttaaaaggtcgtatttttttttttaaaaaagtaaatttgtttcgaaggtaaaggattttttaaagttttttgtgtttttttgttttatttttaaaggattttttgtttttgaaataattttatttttttaagggaaaaaggggggtttttgggggggttagtatttattttttttagttgaaaatatagaatgagtattttgaatttgatttcttccaaaattggccaaaggctaaaaa

SEQ ID NO: 14 - DNA, 296 bp, Artificial Sequence
  Synthetic
acagcaaattcaaatactcatactatatctacaactaaaaaaactaaatactaacaccccaaaaaaccacacttttccccttaaaaaaataaacttatttcaaaaacaaaaaatcctctaaaaataaaacaaaaaaacacaaaaaactctaaaaaatcctctaccttcgaaacaaatttactctcttaaaaaaaaaaatacgaccttttaaaatatcaacacccaactccctcaattataaatacaacacgaataccttaaattcaaactcggggcctactcttcctttctaaaaa